European Patent Specification EP 4 114 843 B1, published August 16, 2023. Title: Method for producing a mammalian brain protein hydrolysate. Applicant: EVER Neuro Pharma GmbH. The sequence listing filed with the application follows.

SEQUENCE LISTING (3 sequences)

SEQ ID NO: 1 - protein, 7 aa, Homo sapiens
NMVPFPR

SEQ ID NO: 2 - protein, 20 aa, Homo sapiens
ASAFQGIGSTHWVYDGVGNS

SEQ ID NO: 3 - protein, 4 aa, Homo sapiens
DLHW